European Patent Application EP 4 772 617 A1, published July 8, 2026. Title: 可静脉注射给药的TPK表达病毒及其治疗阿尔茨海默病的应用. Applicant: 复旦大学附属中山医院. The sequence listing filed with the application follows.

SEQUENCE LISTING (9 sequences)

SEQ ID NO: 1 - DNA, 6074 bp, vector
  source 1..6074: mol_type = genomic DNA
cctgcaggcagctgcgcgctcgctcgctcactgaggccgcccgggcaaagcccgggcgtcgggcgacctttggtcgcccggcctcagtgagcgagcgagcgcgcagagagggagtggccaactccatcactaggggttcctgcggccgcacgcgtgtgtctagactgcagagggccctgcgtatgagtgcaagtgggttttaggaccaggatgaggcggggtgggggtgcctacctgacgaccgaccccgacccactggacaagcacccaacccccattccccaaattgcgcatcccctatcagagagggggaggggaaacaggatgcggcgaggcgcgtgcgcactgccagcttcagcaccgcggacagtgccttcgcccccgcctggcggcgcgcgccaccgccgcctcagcactgaaggcgcgctgacgtcactcgccggtcccccgcaaactccccttcccggccaccttggtcgcgtccgcgccgccgccggcccagccggaccgcaccacgcgaggcgcgagataggggggcacgggcgcgaccatctgcgctgcggcgccggcgactcagcgctgcctcagtctgcggtgggcagcggaggagtcgtgtcgtgcctgagagcgcagtcgagaaggatccgccaccatggagcatgcctttaccccgttggaacccctgctacctacggggaacttgaaatactgccttgtggttcttaatcagcctttggatgcacgatttcgccatctttggaaaaaagctctcttaagagcctgtgctgatgggggtgccaaccacttatatgatctcactgaaggagagagagaaagcttcttgcctgaattcgtcagtggggactttgattctattaggcctgaagtcaaagagtactacaccaagaagggctgtgatcttatttcaactcctgaccaagaccacactgactttaccaagtgtcttcaagtgctccaaaggaagatagaggaaaaggaactgcaggttgacgtgattgtgacactgggaggtctcggtgggcgttttgaccaaatcatggcctctgtgaatacccttttccaagccactcacatcactcctgtgccgattataataatccaaaaggactctctcatctacctcctccaacccgggaagcacaggctccatgtagacactggaatggaagggagctggtgtggcctgattcctgttggacagccttgcaaccaggtgacgacaacaggcctgaaatggaacctcacaaatgatgttcttggctttggaacactggtcagtacttctaacacctacgatgggtccggccttgtcactgtggaaactgaccacccactcctctggaccatggccatcaagagcgtcgacggaagcggagctactaacttcagcctgctgaagcaggctggagacgtggaggagaaccctggacctactagtgccaccatggtgagcaagggcgaggagctgttcaccggggtggtgcccatcctggtcgagctggacggcgacgtaaacggccacaagttcagcgtgtccggcgagggcgagggcgatgccacctacggcaagctgaccctgaagttcatctgcaccaccggcaagctgcccgtgccctggcccaccctcgtgaccaccctgacctacggcgtgcagtgcttcagccgctaccccgaccacatgaagcagcacgacttcttcaagtccgccatgcccgaaggctacgtccaggagcgcaccatcttcttcaaggacgacggcaactacaagacccgcgccgaggtgaagttcgagggcgacaccctggtgaaccgcatcgagctgaagggcatcgacttcaaggaggacggcaacatcctggggcacaagctggagtacaactacaacagccacaacgtctatatcatggccgacaagcagaagaacggcatcaaggtgaacttcaagatccgccacaacatcgaggacggcagcgtgcagctcgccgaccactaccagcagaacacccccatcggcgacggccccgtgctgctgcccgacaaccactacctgagcacccagtccgccctgagcaaagaccccaacgagaagcgcgatcacatggtcctgctggagttcgtgaccgccgccgggatcactctcggcatggacgagctgtacaagtaatagaagcttatcgataatcaacctctggattacaaaatttgtgaaagattgactggtattcttaactatgttgctccttttacgctatgtggatacgctgctttaatgcctttgtatcatgctattgcttcccgtatggctttcattttctcctccttgtataaatcctggttgctgtctctttatgaggagttgtggcccgttgtcaggcaacgtggcgtggtgtgcactgtgtttgctgacgcaacccccactggttggggcattgccaccacctgtcagctcctttccgggactttcgctttccccctccctattgccacggcggaactcatcgccgcctgccttgcccgctgctggacaggggctcggctgttgggcactgacaattccgtggtgttgtcggggaaatcatcgtcctttccttggctgctcgcctatgttgccacctggattctgcgcgggacgtccttctgctacgtcccttcggccctcaatccagcggaccttccttcccgcggcctgctgccggctctgcggcctcttccgcgtcttcgccttcgccctcagacgagtcggatctccctttgggccgcctccccgcatcgataccgagcgctgctcgagagatctacgggtggcatccctgtgacccctccccagtgcctctcctggccctggaagttgccactccagtgcccaccagccttgtcctaataaaattaagttgcatcattttgtctgactaggtgtccttctataatattatggggtggaggggggtggtatggagcaaggggcaagttgggaagacaacctgtagggcctgcggggtctattgggaaccaagctggagtgcagtggcacaatcttggctcactgcaatctccgcctcctgggttcaagcgattctcctgcctcagcctcccgagttgttgggattccaggcatgcatgaccaggctcagctaatttttgtttttttggtagagacggggtttcaccatattggccaggctggtctccaactcctaatctcaggtgatctacccaccttggcctcccaaattgctgggattacaggcgtgaaccactgctcccttccctgtccttctgattttgtaggtaaccacgtgcggaccgagcggccgcaggaacccctagtgatggagttggccactccctctctgcgcgctcgctcgctcactgaggccgggcgaccaaaggtcgcccgacgcccgggctttgcccgggcggcctcagtgagcgagcgagcgcgcagctgcctgcaggggcgcctgatgcggtattttctccttacgcatctgtgcggtatttcacaccgcatacgtcaaagcaaccatagtacgcgccctgtagcggcgcattaagcgcggcgggtgtggtggttacgcgcagcgtgaccgctacacttgccagcgccctagcgcccgctcctttcgctttcttcccttcctttctcgccacgttcgccggctttccccgtcaagctctaaatcgggggctccctttagggttccgatttagtgctttacggcacctcgaccccaaaaaacttgatttgggtgatggttcacgtagtgggccatcgccctgatagacggtttttcgccctttgacgttggagtccacgttctttaatagtggactcttgttccaaactggaacaacactcaaccctatctcgggctattcttttgatttataagggattttgccgatttcggcctattggttaaaaaatgagctgatttaacaaaaatttaacgcgaattttaacaaaatattaacgtttacaattttatggtgcactctcagtacaatctgctctgatgccgcatagttaagccagccccgacacccgccaacacccgctgacgcgccctgacgggcttgtctgctcccggcatccgcttacagacaagctgtgaccgtctccgggagctgcatgtgtcagaggttttcaccgtcatcaccgaaacgcgcgagacgaaagggcctcgtgatacgcctatttttataggttaatgtcatgataataatggtttcttagacgtcaggtggcacttttcggggaaatgtgcgcggaacccctatttgtttatttttctaaatacattcaaatatgtatccgctcatgagacaataaccctgataaatgcttcaataatattgaaaaaggaagagtatgagtattcaacatttccgtgtcgcccttattcccttttttgcggcattttgccttcctgtttttgctcacccagaaacgctggtgaaagtaaaagatgctgaagatcagttgggtgcacgagtgggttacatcgaactggatctcaacagcggtaagatccttgagagttttcgccccgaagaacgttttccaatgatgagcacttttaaagttctgctatgtggcgcggtattatcccgtattgacgccgggcaagagcaactcggtcgccgcatacactattctcagaatgacttggttgagtactcaccagtcacagaaaagcatcttacggatggcatgacagtaagagaattatgcagtgctgccataaccatgagtgataacactgcggccaacttacttctgacaacgatcggaggaccgaaggagctaaccgcttttttgcacaacatgggggatcatgtaactcgccttgatcgttgggaaccggagctgaatgaagccataccaaacgacgagcgtgacaccacgatgcctgtagcaatggcaacaacgttgcgcaaactattaactggcgaactacttactctagcttcccggcaacaattaatagactggatggaggcggataaagttgcaggaccacttctgcgctcggcccttccggctggctggtttattgctgataaatctggagccggtgagcgtgggtctcgcggtatcattgcagcactggggccagatggtaagccctcccgtatcgtagttatctacacgacggggagtcaggcaactatggatgaacgaaatagacagatcgctgagataggtgcctcactgattaagcattggtaactgtcagaccaagtttactcatatatactttagattgatttaaaacttcatttttaatttaaaaggatctaggtgaagatcctttttgataatctcatgaccaaaatcccttaacgtgagttttcgttccactgagcgtcagaccccgtagaaaagatcaaaggatcttcttgagatcctttttttctgcgcgtaatctgctgcttgcaaacaaaaaaaccaccgctaccagcggtggtttgtttgccggatcaagagctaccaactctttttccgaaggtaactggcttcagcagagcgcagataccaaatactgtccttctagtgtagccgtagttaggccaccacttcaagaactctgtagcaccgcctacatacctcgctctgctaatcctgttaccagtggctgctgccagtggcgataagtcgtgtcttaccgggttggactcaagacgatagttaccggataaggcgcagcggtcgggctgaacggggggttcgtgcacacagcccagcttggagcgaacgacctacaccgaactgagatacctacagcgtgagctatgagaaagcgccacgcttcccgaagggagaaaggcggacaggtatccggtaagcggcagggtcggaacaggagagcgcacgagggagcttccagggggaaacgcctggtatctttatagtcctgtcgggtttcgccacctctgacttgagcgtcgatttttgtgatgctcgtcaggggggcggagcctatggaaaaacgccagcaacgcggcctttttacggttcctggccttttgctggccttttgctcacatgt

SEQ ID NO: 2 - DNA, 448 bp, promoter
  source 1..448: mol_type = other DNA
agtgcaagtgggttttaggaccaggatgaggcggggtgggggtgcctacctgacgaccgaccccgacccactggacaagcacccaacccccattccccaaattgcgcatcccctatcagagagggggaggggaaacaggatgcggcgaggcgcgtgcgcactgccagcttcagcaccgcggacagtgccttcgcccccgcctggcggcgcgcgccaccgccgcctcagcactgaaggcgcgctgacgtcactcgccggtcccccgcaaactccccttcccggccaccttggtcgcgtccgcgccgccgccggcccagccggaccgcaccacgcgaggcgcgagataggggggcacgggcgcgaccatctgcgctgcggcgccggcgactcagcgctgcctcagtctgcggtgggcagcggaggagtcgtgtcgtgcctgagagcgcag

SEQ ID NO: 3 - DNA, 729 bp, gene
  source 1..729: mol_type = other DNA
atggagcatgcctttaccccgttggaacccctgctacctacggggaacttgaaatactgccttgtggttcttaatcagcctttggatgcacgatttcgccatctttggaaaaaagctctcttaagagcctgtgctgatgggggtgccaaccacttatatgatctcactgaaggagagagagaaagcttcttgcctgaattcgtcagtggggactttgattctattaggcctgaagtcaaagagtactacaccaagaagggctgtgatcttatttcaactcctgaccaagaccacactgactttaccaagtgtcttcaagtgctccaaaggaagatagaggaaaaggaactgcaggttgacgtgattgtgacactgggaggtctcggtgggcgttttgaccaaatcatggcctctgtgaatacccttttccaagccactcacatcactcctgtgccgattataataatccaaaaggactctctcatctacctcctccaacccgggaagcacaggctccatgtagacactggaatggaagggagctggtgtggcctgattcctgttggacagccttgcaaccaggtgacgacaacaggcctgaaatggaacctcacaaatgatgttcttggctttggaacactggtcagtacttctaacacctacgatgggtccggccttgtcactgtggaaactgaccacccactcctctggaccatggccatcaagagc

SEQ ID NO: 4 - DNA, 589 bp, unidentified
  source 1..589: mol_type = other DNA
aatcaacctctggattacaaaatttgtgaaagattgactggtattcttaactatgttgctccttttacgctatgtggatacgctgctttaatgcctttgtatcatgctattgcttcccgtatggctttcattttctcctccttgtataaatcctggttgctgtctctttatgaggagttgtggcccgttgtcaggcaacgtggcgtggtgtgcactgtgtttgctgacgcaacccccactggttggggcattgccaccacctgtcagctcctttccgggactttcgctttccccctccctattgccacggcggaactcatcgccgcctgccttgcccgctgctggacaggggctcggctgttgggcactgacaattccgtggtgttgtcggggaaatcatcgtcctttccttggctgctcgcctatgttgccacctggattctgcgcgggacgtccttctgctacgtcccttcggccctcaatccagcggaccttccttcccgcggcctgctgccggctctgcggcctcttccgcgtcttcgccttcgccctcagacgagtcggatctccctttgggccgcctccccgc

SEQ ID NO: 5 - DNA, 46 bp, Primer
  source 1..46: mol_type = unassigned DNA
agcgcagtcgagaaggatccgccaccatggagcatgcctttacccc

SEQ ID NO: 6 - DNA, 40 bp, primer
  source 1..40: mol_type = unassigned DNA
gtagctccgcttccgtcgacgctcttgatggccatggtcc

SEQ ID NO: 7 - DNA, 17 bp, Primer
  source 1..17: mol_type = unassigned DNA
gcgctgcctcagtctgc

SEQ ID NO: 8 - DNA, 22 bp, Primer
  source 1..22: mol_type = other DNA
cgtcgccgtccagctcgaccag

SEQ ID NO: 9 - protein, 19 aa, peptide
ATNFSLLKQAGDVEENPGP